European Patent Application EP 4 286 534 A1, published December 6, 2023. Title: A method of determining the likelihood of a horse to race. Applicant: PLUSVITAL LTD. The sequence listing filed with the application follows.

SEQUENCE LISTING (9 sequences)

SEQ ID NO: 1 - DNA, 84 bp, Unknown
  Synthetic sequence
tggaccgagacaaacagattggttctaatatgagtcgggttcgcagacagattgtgagcaaagggacatgctctcctttggact

SEQ ID NO: 2 - DNA, 84 bp, Unknown
  Synthetic sequence
tgaaccgagacaaacagattggccttaatataaactgggtcagcagacagattgtgaacaaaggggtacatcattctttggact

SEQ ID NO: 3 - DNA, 84 bp, Unknown
  Synthetic sequence
cgggccgggaaagacaaacctgccttaatataaactaggtccatgggcgaattataggagaagggacgtgctctcctttggact

SEQ ID NO: 4 - DNA, 84 bp, Unknown
  Synthetic sequence
cggaccgagacaaaaagattggcctcggcagacgtcgtgcccacagacaagttatgagaaagagaacacaccatttccggaact

SEQ ID NO: 5 - DNA, 84 bp, Unknown
  Synthetic sequence
tggaccaagacaaacagattggttctggcagaagccgggtccatagataaaccgggggaggaaagacacaccatccttttgact

SEQ ID NO: 6 - DNA, 84 bp, Unknown
  Synthetic sequence
tggaatgatgagggccggcctgttctggtgtacgtcggatccataaacggaccgggagaaagagaacacaccatttccggaact

SEQ ID NO: 7 - DNA, 84 bp, Unknown
  Synthetic sequence
tagaatgatgagggccggcctattctaatatgagtcggatcagcagacagattgtaggagaagggacgtgctctcttctggact

SEQ ID NO: 8 - DNA, 84 bp, Unknown
  Synthetic sequence
tggaccgagacaaaaagattggcctcggcagacgtcgggtccatagataaaccgggggaggaaagacatgttagttcctgactc

SEQ ID NO: 9 - DNA, 84 bp, Unknown
  Synthetic sequence
cgggccgggaaagacaaacctattctaatatgagtcggatcagcagacagattgtaggagaagggacgcaccatttccggaact